European Patent Specification EP 3 999 665 B1, published May 10, 2023. Title: Method for determining the risk of an avian pathogenic E. coli (APEC) infection in an avian flock. Applicant: Evonik Operations GmbH. The sequence listing filed with the application follows.

SEQUENCE LISTING (24 sequences)

SEQ ID NO: 1 - DNA, 2178 bp, Escherichia coli
atgagaattaacaaaatcctctggtcgctaactgtgctcctggttgggttgaatagccaggtatcagtagccaaatcctccgacgatgataatgacgagactctggtggtggaagccaccgctgagcaggtattaaaacagcagccgggcgtgtcggttattaccagcgaggatattaaaaagacccctccggtaaacgacctttcagatattattcgtaaaatgcctggcgtcaatcttaccggcaatagcgcctcgggcacacgcggtaacaaccgccagatcgatattcgtggtatggggccggaaaacaccttaattttaattgatggtgtaccggtgacgtcacgtaactccgtgcgttatagctggcgtggagagcgtgatacccgcggtgacaccaactgggtgccaccggaacaggttgagcgtattgaagtgatccgcggccctgcggcggcgcgctacggttcgggggcagccgggggggtggtgaacatcattaccaaacgtcccaccaacgactggcacggttcgctgtcgttatacaccaatcagccggaaagtagcgatgagggcgctacgcgtcgcgccaatttcagccttagtgggcctctggctggtaatgctcttaccacgcgtttgtatggtaacctgaataaaacggatgctgacagttgggatattaattctccggtcggtacgaaaaacgcagccgggcatgaaggggtacgtaacaaagatattaacggcgttgtctcgtggaaattaaatccgcagcagattctcgatttcgaagccggatatagccgccaggggaatatctatgcgggcgatacgcaaaacagttcttccagtgcagttaccgaaagcctggcaaaatccggcaaagagacgaaccgcctgtaccgacagaattatggcattacgcataatggtatctgggactggggacaaagtcgctttggtgtttattacgagaaaaccaataatacccgcatgaatgaaggattatccggcggtggtgaagggcgtattttagcgggtgaaaagtttacgaccaatcgcctgagttcctggcgaaccagcggcgagcttaatattcctttgaatgtgatggttgatcaaacgctgaccgttggtgcagagtggaaccgcgataagctcgatgatccttcctctaccagcctgacggtgaatgacagtgatatcagcggtatttctggctctgctgcggatcgcagcagtaaaaatcattctcaaatcagtgcgctgtatattgaagataacattgagccggttcctggcacgaatatcattcccggcctgcgctttgattatctcagcgactccggcgggaacttcagccccagtctgaatctttcgcaggaattgggcgattatttcaaagtcaaagcaggggttgcccgaacctttaaagctccaaacctgtatcaatccagtgaaggctatctgctctactcgaaaggcaatggctgtccaaaagatattacatcaggcgggtgctacctgatcggtaataaagatctcgatccggaaatcagcgtcaataaagaaattgggctggagttcacctgggaagattaccacgcaagtgtgacctacttccgcaatgattaccagaataagatcgtggccggggataacgttatcgggcaaaccgcttcaggcgcatatatcctcaagtggcagaatggcgggaaagctctggtggacggtatcgaagccagtatgtctttcccactggtgaaagatcgtctgaactggaataccaatgccacatggatgatcacttcggagcaaaaagacaccggtaatcctctgtcggtcatcccgaaatatactatcaataactcgcttaactggaccatcacccaggcgttttctgccagcgtcaactggacgttatatggcagacaaaaaccgcgtactcatgcggaaacccgcagtgaagatactggcggtctgtcaggtaaagagctgggcgcttattcactggtggggacgaacttcaattacgatattaataaaaatctgcgtcttaatgtcggcgtcagtaatatcctcaataaacagatcttccgatcttctgaaggggcgaatacctataacgagccaggccgggcttactatgccggagttaccgcatcattctga

SEQ ID NO: 2 - DNA, 954 bp, Escherichia coli
atgtacttaaagattcttgctactgcactctcagctcctgtagcgtttgctgcactggcttctgatactgggctttcttttacaccggagaaaatcagtacggagattgattttggcactttaagtggcaaggccaaagaacgggtttatctgcctgaagaaaaagggcgcaaagccagccagctggactggaaatacagtaatgcgccaattgtcaagggggcatttaactgggatctgttacccagagtatctgtcggtgcctcagggtggacaacattagctggtcgtggaggcaatatggtggacagggactggctggatacgagcaatcccggaacctggactgatgagagtaaacatccgaatacccgtctaaattttgctaatgaattcgacctgaatattaagggatggctcctgaatcaaccagactatcagttaggtcttatggctggttaccaggaaaatcgttatagctttacagcaaaaggaggctcttatatctatagtagtgagggaggcttccgggatgaaacgggatcatttccagatggtgaaagagctataggctacaaacaacactttaaaatgccctatatagggttaaccggtaattatcggtatgatagctttgagttcggggggagtttcaaatatagcggatgggtgaaggcatcggataatgatgagcattacaaccctgagaaaaggatcacctatcgtagcgatgtaaataatcagaactattactctgtctcactacatgctggttattatattacacctgcagctaaagtttatgtcgaaggaacatggaaccgtattactaataagaaaggtgatacttctctgtactccagaaatttgaatatatctgatcacaccaaaaatggtgcaggcattgaaagctataactttatgaccacagctggtctgaagtattatttttaa

SEQ ID NO: 3 - DNA, 1109 bp, Escherichia coli
tgaaattattattacttacaggtgcaacaggatttcttggtggcgcggtcctggataagctgctggataactgtaataatataaatttgctacttttagtacgagcacctactccacaagcgggactggaaagaattaaagaaaatatgcgtaaatttaatgtttgtgaggaaaggttgcatgcattaactaatgataacatcttgcctggggatctaaataatccggaagcctttctcatggatcctcgtcttgatgaagtcactcatgttataaactgtgcggctatagcttcttttggtaataatccttttatatggaatgtgaatgttacaggtacacttgcttttgcaagaagaatggcaaaagtggcaggactgaaacgcttccttcatgttggtactgctatgtcttgtacacctcatacggggtcgctagttaaggaagagtctgcttcatcagaaacaggtgaacatttagtggagtatacgcattcaaaagcaacaatagaatatctgatgcgtaagcagtgtcctgatttacctttgttggttgcccgaccatcaattattgttggccacagtcgtttagggtgcttaccttcaaccagtattttctgggtattcagaatggggttaatgttgcaaaaatttatgtgctctctggatgataaaatagatgttatccctgtagattattgtgctgatgcattgctaatgttgcttgaaagctcgttaattaatggtgagattgttcatatatcagcaggtaaagaaagtagtgtgacgttctctgctattgacgaagctgtagcccgtgctttgaactgtgatcctgttggagacagatatactaaagtcagttatgacatactggcaatgagccgtcatgattttaaaaatatttttggtccctgtaacgaacgccttatgttaaaagccattcgtttatatggagcgttcagtatgctcaatgtttgtttcagtaacgacaagctactgagtatcggaatgcctaaaccgccaaagtttactgattatattaaatactgtatagaaacgacaaaacacctttcaattcaacaacaaatggaagttgattttaaataa

SEQ ID NO: 4 - DNA, 309 bp, Escherichia coli
atgcaggataataagatgaaaaaaatgttattttctgccgctctggcaatgcttattacaggatgtgctcaacaaacgtttactgttggaaacaaaccgacagcagtaacaccaaaggaaaccatcactcatcatttcttcgtttcgggaattggacaagagaaaactgttgatgcagccaaaatttgtggcggtgcagaaaatgttgttaaaacagaaactcagcaaacattcgtaaatggattgctcggttttatcacttttggcatctatactccgctggaagcccgggtatattgctcacaatag

SEQ ID NO: 5 - DNA, 2202 bp, Escherichia coli
atgatgataagcaaaaagtatacgctttgggctctcaacccactgcttcttaccatgatggcgccagcagtcgctcaacaaaccgatgatgaaacgttcgtggtgtctgccaaccgcagcaatcgcaccgtagcggagatggcgcaaaccacctgggttatcgaaaacgccgaactggaacagcagattcagggcggcaaagagcttaaagacgcactggctcagctgatccctggccttgacgtcagcagccggagccgcaccaactacggtatgaatgtgcgtggccgcccgctggtcgtgctggttgacggcgtgcgtctcaactcttcacgtaccgacagccgacaactggactctatagatccttttaatatcgaccatattgaagtgatctccggtgcgacgtccctgtacggcggcggcagtaccggtggcctgatcaacatcgtgaccaaaaaaggccagccggaaaccatgatggagtttgaggctggcaccaaaagtggctttagcagcagtaaagatcacgatgaacgcattgccggagctgtctccggcggaaatgagcatatctccggacgtctttccgtggcatatcagaaatttggcggctggtttgacggtaacggcgatgccaccttgcttgataacacccagaccggcctgcagtactccgatcggctggacatcatgggaactggtacgctgaacatcgatgaatcccggcagcttcagttgatcacacagtactataaaagccagggcgacgacgattacgggcttaatctcgggaaaggcttctctgccatcagagggaccagcacgccattcgtcagtaacgggctgaattccgaccgtattcccggcactgagcggcatttgatcagcctgcagtactctgacagcgcttttctgggacaggagctggtcggtcaggtttactaccgcgatgagtcgttgcgattctacccgttcccgacggtaaatgcgaacaaacaggtgacggctttctcttcgtcacagcaggacaccgaccagtacggcatgaaactgactctgaacagcaaaccgatggacggctggcaaatcacctgggggctggatgctgatcatgagcgctttacctccaaccagatgttcttcgacctggctcaggcaagcgcttccggagggctgaacaacaagaagatttacaccaccgggcgctatccgtcgtatgacatcaccaacctggcggccttcctgcaatcaggctatgacatcaataatctctttaccctcaacggtggcgtacgctatcagtacactgaaaacaagattgatgatttcatcggctacgcgcagcaacggcagattgccgccgggaaggctacatccgccgacgccattcctggcggctcagtcgattacgacaacttcctgttcaacgccggtctgctgatgcacatcaccgaacgccagcaggcatggctcaacttctcccagggcgtggagctgccggacccgggtaaatactatggtcgcggcatctatggtgctgcagtgaacggccatcttcctctaacaaagagtgtgaacgtcagcgacagcaagctggaaggcgtgaaagtcgattcttatgagctgggctggcgctttactggcaataatctgcgtacccaaatcgcggcctactattcgatttctgataagagcgtggtggcgaataaagatctgaccatcagcgtggtggacgacaaacgccgtatttacggcgtggaaggtgcggtggactacctgattcctgatactgactggagtaccggagtgaacttcaacgtgctgaaaactgagtcgaaagtgaacggtacctggcagaaatacgatgtgaagacagcaagcccatcaaaagcgacagcctacattggctgggcaccggacccgtggagtctgcgcgtgcagagcaccacctcctttgacgtgagcgacgcgcagggctacaaggtcgatggctataccaccgtggatctgctcggcagttatcagcttccggtgggtacactcagcttcagcattgaaaaccttttcgaccgtgactacaccactgtctgggggcagcgtgcaccactgtactacagcccgggttacggcccagcgtcactgtacgactacaaaggcaggggccgaacctttggtctgaactactctgtgctgttctga

SEQ ID NO: 6 - DNA, 1455 bp, Escherichia coli
atggaacatcagagaaaactattccagcaacgcggctatagcgaagatctattgccgaaaacgcaaagccagcggacctggaaaacatttaactattttaccttatggatgggttcggttcataacgttcccaattatgtgatggtcggcggcttttttattctcggcttgtctacctttagtattatgctggcaattatcctcagcgcctttttcattgccgcggtaatggtattaaacggtgctgcgggcagtaaatacggtgtgccttttgccatgatcctgcgtgcttcttacggtgtacgtggtgcactgtttcccggattattaaggggcggaattgccgccatcatgtggtttggtttgcaatgttacgcggggtcactggcctgcttgattctgattggcaaaatctggccgggatttttaactctcggtggtgatttcactctgttaggcctttctctaccgggcttaattactttcttaatcttctggctggtcaacgttggtataggttttggcggtggcaaagttttaaataaattcactgccattcttaacccgtgcatctatatcgttttcggcggtatggcgatttgggcgatttcactggtcgggatcggtccaatctttgactacattccgagcggtattcagaaagcagaaaacggtggcttcctgttcctggtggtgattaacgcggtagttgcggtctgggcggcaccggcggtgagcgcatccgactttacgcaaaacgcccactcgtttcgtgagcaggcgctggggcaaacgctgggtttagttgtggcctatattctgtttgcggtcgccggggtatgtattattgccggagccagtattcactacggcgctgatacctggaacgtgctggatattgttcagcgttgggacagcctgttcgcctcgttctttgcggtactggttattctgatgacaactatctccactaacgcgaccggtaatattattccagccggttatcagattgccgccattgcaccgacaaaactgacctataaaaacggcgtactgattgccagtattatcagcttgctgatctgcccgtggaaattaatggaaaatcaggacagcatttatcttttcctcgatattatcggcggaatgcttggtccggtaattggtgtcatgatggcgcattattttgtggtgatgcgcggacaaattaatcttgatgaactgtataccgcacctggcgattataaatattacgataacggttttaacctcactgcgttttcagtaactctggtggccgttattttatctcttggcggtaagtttattcactttatggaaccgttatcgcgtgtttcatggtttgtcggcgtcatcgtcgcctttgcggcctacgccttattaaagaaacgtacaacagcagaaaaaacaggagagcaaaaaaccataggttaa

SEQ ID NO: 7 - DNA, 25 bp, artificial
  Primer
aatccggcaaagagacgaaccgcct

SEQ ID NO: 8 - DNA, 26 bp, artificial
  Primer
gttcgggcaacccctgctttgacttt

SEQ ID NO: 9 - DNA, 28 bp, artificial
  Primer
tcatcccggaagcctccctcactactat

SEQ ID NO: 10 - DNA, 28 bp, artificial
  Primer
tagcgtttgctgcactggcttctgatac

SEQ ID NO: 11 - DNA, 26 bp, artificial
  Primer
ggccacagtcgtttagggtgcttacc

SEQ ID NO: 12 - DNA, 26 bp, artificial
  Primer
ggcggtttaggcattccgatactcag

SEQ ID NO: 13 - DNA, 22 bp, artificial
  Primer
cagcaacccgaaccacttgatg

SEQ ID NO: 14 - DNA, 21 bp, artificial
  Primer
agcattgccagagcggcagaa

SEQ ID NO: 15 - DNA, 22 bp, artificial
  Primer
ggctggacatcatgggaactgg

SEQ ID NO: 16 - DNA, 21 bp, artificial
  Primer
cgtcgggaacgggtagaatcg

SEQ ID NO: 17 - DNA, 20 bp, artificial
  Primer
gcgcactgatttgagaatga

SEQ ID NO: 18 - DNA, 20 bp, artificial
  Primer
cttcctctaccagcctgacg

SEQ ID NO: 19 - DNA, 20 bp, artificial
  Probe
cgatccgcagcagagccaga

SEQ ID NO: 20 - DNA, 20 bp, artificial
  Primer
cgggaattggacaagagaaa

SEQ ID NO: 21 - DNA, 20 bp, artificial
  Primer
atatacccgggcttccaaac

SEQ ID NO: 22 - DNA, 22 bp, artificial
  Probe
atgcagccaaaatttgtggcgg

SEQ ID NO: 23 - DNA, 20 bp, artificial
  Primer
tgattggcaaaatctggccg

SEQ ID NO: 24 - DNA, 20 bp, artificial
  Primer
gaaatcgcccaaatcgccat